European Patent Application EP 4 491 190 A1, published January 15, 2025. Title: Small proteins for use as senolytic and senomorphic agents. Applicant: FUNDACION IMDEA ALIMENTACION. The sequence listing filed with the application follows.

SEQUENCE LISTING (4 sequences)

SEQ ID NO: 1 - protein, 176 aa, Stichodactyla helianthus
SELAGTIIDGASLTFEVLDKVLGELGKVSRKIAVGIDNESGGTWTALNAYFRSGTTDVILPEVVPNTKALLYSGRKSSGPVATGAVAAFAYYMSNGNTLGVMFSVPFDYNWYSNWWDVKIYPGKRRADQGMYEDMYYGNPYRGDNGWYQKNLGYGLRMKGIMTSAGEAKMQIKISR

SEQ ID NO: 2 - protein, 183 aa, synthetic construct
MSELAGTIIDGASLTFEVLDKVLGELGKVSRKIAVGIDNESGGTWTALNAYFRSGTTDVILPEVVPNTKALLYSGRKSSGPVATGAVAAFAYYMSNGNTLGVMFSVPFDYNWYSNWWDVKIYPGKRRADQGMYEDMYYGNPYRGDNGWYQKNLGYGLRMKGIMTSAGEAKMQIKISRHHHHHH

SEQ ID NO: 3 - protein, 175 aa, Stichodactyla helianthus [sequence omitted]

SEQ ID NO: 4 - protein, 176 aa, Stichodactyla helianthus
SALAGTIIAGASLTFEVLDKVLGELGKVSRKIAVGIDNESGGTWTALNAYFRSGTTDVILPEVVPNTKALLYSGRKSSGPVATGAVAAFAYYMSNGNTLGVMFSVPFDYNWYSNWWDVKIYPGKRRADQGMYEDMYYGNPYRGDNGWYQKNLGYGLRMKGIMTSAGEAKMQIKISR